European Patent Application EP 4 253 423 A1, published October 4, 2023. Title: BISPECIFIC RECOMBINANT PROTEIN AND USE THEREOF. Applicant: SHANGHAI LYN-CREST ENTERPRISE MANAGEMENT CO., LTD. The sequence listing filed with the application follows.

SEQUENCE LISTING (64 sequences)

SEQ ID NO: 1 - protein, 452 aa, Artificial Sequence
  Ofatumumab(H)-Fc1
EVQLVESGGGLVQPGRSLRLSCAASGFTFNDYAMHWVRQAPGKGLEWVSTISWNSGSIGYADSVKGRFTISRDNAKKSLYLQMNSLRAEDTALYYCAKDIQYGNYYYGMDVWGQGTTVTVSSASTKGPSVFPLAPSSKSTSGGTAALGCLVKDYFPEPVTVSWNSGALTSGVHTFPAVLQSSGLYSLSSVVTVPSSSLGTQTYICNVNHKPSNTKVDKKVEPKSCDKTHTCPPCPAPELLGGPSVFLFPPKPKDTLMISRTPEVTCVVVDVSHEDPEVKFNWYVDGVEVHNAKTKPREEQYNSTYRVVSVLTVLHQDWLNGKEYKCKVSNKALPAPIEKTISKAKGQPREPQVYTLPPSRDELTKNQVSLSCAVKGFYPSDIAVEWESNGQPENNYKTTPPVLDSDGSFFLVSKLTVDKSRWQQGNVFSCSVMHEALHNHYTQKSLSLSPGK

SEQ ID NO: 2 - protein, 558 aa, Artificial Sequence
  Ofatumumab(L)-SIRPD1-Fc2
EIVLTQSPATLSLSPGERATLSCRASQSVSSYLAWYQQKPGQAPRLLIYDASNRATGIPARFSGSGSGTDFTLTISSLEPEDFAVYYCQQRSNWPITFGQGTRLEIKRTVAAPSVFIFPPSDEQLKSGTASVVCLLNNFYPREAKVQWKVDNALQSGNSQESVTEQDSKDSTYSLSSTLTLSKADYEKHKVYACEVTHQGLSSPVTKSFNRGECEEELQVIQPDKSVSVAAGESAILHCTVTSLIPVGPIQWFRGAGPARELIYNQKEGHFPRVTTVSESTKRENMDFSISISAITPADAGTYYCVKFRKGSPDTEFKSGAGTELSVRAKPDKTHTCPPCPAPELLGGPSVFLFPPKPKDTLMISRTPEVTCVVVDVSHEDPEVKFNWYVDGVEVHNAKTKPREEQYNSTYRVVSVLTVLHQDWLNGKEYKCKVSNKALPAPIEKTISKAKGQPREPQVYTLPPSRDELTKNQVSLWCLVKGFYPSDIAVEWESNGQPENNYKTTPPVLDSDGSFFLYSKLTVDKSRWQQGNVFSCSVMHEALHNHYTQKSLSLSPGK

SEQ ID NO: 3 - protein, 573 aa, Artificial Sequence
  Ofatumumab(L)-(GGGGS)3-SIRPD1-Fc2
EIVLTQSPATLSLSPGERATLSCRASQSVSSYLAWYQQKPGQAPRLLIYDASNRATGIPARFSGSGSGTDFTLTISSLEPEDFAVYYCQQRSNWPITFGQGTRLEIKRTVAAPSVFIFPPSDEQLKSGTASVVCLLNNFYPREAKVQWKVDNALQSGNSQESVTEQDSKDSTYSLSSTLTLSKADYEKHKVYACEVTHQGLSSPVTKSFNRGECGGGGSGGGGSGGGGSEEELQVIQPDKSVSVAAGESAILHCTVTSLIPVGPIQWFRGAGPARELIYNQKEGHFPRVTTVSESTKRENMDFSISISAITPADAGTYYCVKFRKGSPDTEFKSGAGTELSVRAKPDKTHTCPPCPAPELLGGPSVFLFPPKPKDTLMISRTPEVTCVVVDVSHEDPEVKFNWYVDGVEVHNAKTKPREEQYNSTYRVVSVLTVLHQDWLNGKEYKCKVSNKALPAPIEKTISKAKGQPREPQVYTLPPSRDELTKNQVSLWCLVKGFYPSDIAVEWESNGQPENNYKTTPPVLDSDGSFFLYSKLTVDKSRWQQGNVFSCSVMHEALHNHYTQKSLSLSPGK

SEQ ID NO: 4 - protein, 445 aa, Artificial Sequence
  GC33(H)-Fc1
QVQLVQSGAEVKKPGASVKVSCKASGYTFTDYEMHWVRQAPGQGLEWMGALDPKTGDTAYSQKFKGRVTLTADKSTSTAYMELSSLTSEDTAVYYCTRFYSYTYWGQGTLVTVSSASTKGPSVFPLAPSSKSTSGGTAALGCLVKDYFPEPVTVSWNSGALTSGVHTFPAVLQSSGLYSLSSVVTVPSSSLGTQTYICNVNHKPSNTKVDKKVEPKSCDKTHTCPPCPAPELLGGPSVFLFPPKPKDTLMISRTPEVTCVVVDVSHEDPEVKFNWYVDGVEVHNAKTKPREEQYNSTYRVVSVLTVLHQDWLNGKEYKCKVSNKALPAPIEKTISKAKGQPREPQVYTLPPSRDELTKNQVSLSCAVKGFYPSDIAVEWESNGQPENNYKTTPPVLDSDGSFFLVSKLTVDKSRWQQGNVFSCSVMHEALHNHYTQKSLSLSPGK

SEQ ID NO: 5 - protein, 616 aa, Artificial Sequence
  GC33(L)-(GGGGS)1-IFN 2b-Fc2
DVVMTQSPLSLPVTPGEPASISCRSSQSLVHSNRNTYLHWYLQKPGQSPQLLIYKVSNRFSGVPDRFSGSGSGTDFTLKISRVEAEDVGVYYCSQNTHVPPTFGQGTKLEIKRTVAAPSVFIFPPSDEQLKSGTASVVCLLNNFYPREAKVQWKVDNALQSGNSQESVTEQDSKDSTYSLSSTLTLSKADYEKHKVYACEVTHQGLSSPVTKSFNRGECGGGGSCDLPQTHSLGSRRTLMLLAQMRRISLFSCLKDRHDFGFPQEEFGNQFQKAETIPVLHEMIQQIFNLFSTKDSSAAWDETLLDKFYTELYQQLNDLEACVIQGVGVTETPLMKEDSILAVRKYFQRITLYLKEKKYSPCAWEVVRAEIMRSFSLSTNLQESLRSKEDKTHTCPPCPAPELLGGPSVFLFPPKPKDTLMISRTPEVTCVVVDVSHEDPEVKFNWYVDGVEVHNAKTKPREEQYNSTYRVVSVLTVLHQDWLNGKEYKCKVSNKALPAPIEKTISKAKGQPREPQVYTLPPSRDELTKNQVSLWCLVKGFYPSDIAVEWESNGQPENNYKTTPPVLDSDGSFFLYSKLTVDKSRWQQGNVFSCSVMHEALHNHYTQKSLSLSPGK

SEQ ID NO: 6 - protein, 621 aa, Artificial Sequence
  GC33(L)-(GGGGS)2-IFN 2b-Fc2
DVVMTQSPLSLPVTPGEPASISCRSSQSLVHSNRNTYLHWYLQKPGQSPQLLIYKVSNRFSGVPDRFSGSGSGTDFTLKISRVEAEDVGVYYCSQNTHVPPTFGQGTKLEIKRTVAAPSVFIFPPSDEQLKSGTASVVCLLNNFYPREAKVQWKVDNALQSGNSQESVTEQDSKDSTYSLSSTLTLSKADYEKHKVYACEVTHQGLSSPVTKSFNRGECGGGGSGGGGSCDLPQTHSLGSRRTLMLLAQMRRISLFSCLKDRHDFGFPQEEFGNQFQKAETIPVLHEMIQQIFNLFSTKDSSAAWDETLLDKFYTELYQQLNDLEACVIQGVGVTETPLMKEDSILAVRKYFQRITLYLKEKKYSPCAWEVVRAEIMRSFSLSTNLQESLRSKEDKTHTCPPCPAPELLGGPSVFLFPPKPKDTLMISRTPEVTCVVVDVSHEDPEVKFNWYVDGVEVHNAKTKPREEQYNSTYRVVSVLTVLHQDWLNGKEYKCKVSNKALPAPIEKTISKAKGQPREPQVYTLPPSRDELTKNQVSLWCLVKGFYPSDIAVEWESNGQPENNYKTTPPVLDSDGSFFLYSKLTVDKSRWQQGNVFSCSVMHEALHNHYTQKSLSLSPGK

SEQ ID NO: 7 - protein, 631 aa, Artificial Sequence
  GC33(L)-(GGGGS)4-IFN 2b-Fc2
DVVMTQSPLSLPVTPGEPASISCRSSQSLVHSNRNTYLHWYLQKPGQSPQLLIYKVSNRFSGVPDRFSGSGSGTDFTLKISRVEAEDVGVYYCSQNTHVPPTFGQGTKLEIKRTVAAPSVFIFPPSDEQLKSGTASVVCLLNNFYPREAKVQWKVDNALQSGNSQESVTEQDSKDSTYSLSSTLTLSKADYEKHKVYACEVTHQGLSSPVTKSFNRGECGGGGSGGGGSGGGGSGGGGSCDLPQTHSLGSRRTLMLLAQMRRISLFSCLKDRHDFGFPQEEFGNQFQKAETIPVLHEMIQQIFNLFSTKDSSAAWDETLLDKFYTELYQQLNDLEACVIQGVGVTETPLMKEDSILAVRKYFQRITLYLKEKKYSPCAWEVVRAEIMRSFSLSTNLQESLRSKEDKTHTCPPCPAPELLGGPSVFLFPPKPKDTLMISRTPEVTCVVVDVSHEDPEVKFNWYVDGVEVHNAKTKPREEQYNSTYRVVSVLTVLHQDWLNGKEYKCKVSNKALPAPIEKTISKAKGQPREPQVYTLPPSRDELTKNQVSLWCLVKGFYPSDIAVEWESNGQPENNYKTTPPVLDSDGSFFLYSKLTVDKSRWQQGNVFSCSVMHEALHNHYTQKSLSLSPGK

SEQ ID NO: 8 - protein, 621 aa, Artificial Sequence
  GC33(L)-(GGGGS)2-IFN 2bL26A-Fc2
DVVMTQSPLSLPVTPGEPASISCRSSQSLVHSNRNTYLHWYLQKPGQSPQLLIYKVSNRFSGVPDRFSGSGSGTDFTLKISRVEAEDVGVYYCSQNTHVPPTFGQGTKLEIKRTVAAPSVFIFPPSDEQLKSGTASVVCLLNNFYPREAKVQWKVDNALQSGNSQESVTEQDSKDSTYSLSSTLTLSKADYEKHKVYACEVTHQGLSSPVTKSFNRGECGGGGSGGGGSCDLPQTHSLGSRRTLMLLAQMRRISAFSCLKDRHDFGFPQEEFGNQFQKAETIPVLHEMIQQIFNLFSTKDSSAAWDETLLDKFYTELYQQLNDLEACVIQGVGVTETPLMKEDSILAVRKYFQRITLYLKEKKYSPCAWEVVRAEIMRSFSLSTNLQESLRSKEDKTHTCPPCPAPELLGGPSVFLFPPKPKDTLMISRTPEVTCVVVDVSHEDPEVKFNWYVDGVEVHNAKTKPREEQYNSTYRVVSVLTVLHQDWLNGKEYKCKVSNKALPAPIEKTISKAKGQPREPQVYTLPPSRDELTKNQVSLWCLVKGFYPSDIAVEWESNGQPENNYKTTPPVLDSDGSFFLYSKLTVDKSRWQQGNVFSCSVMHEALHNHYTQKSLSLSPGK

SEQ ID NO: 9 - protein, 621 aa, Artificial Sequence
  GC33(L)-(GGGGS)2-IFN 2bL30A-Fc2
DVVMTQSPLSLPVTPGEPASISCRSSQSLVHSNRNTYLHWYLQKPGQSPQLLIYKVSNRFSGVPDRFSGSGSGTDFTLKISRVEAEDVGVYYCSQNTHVPPTFGQGTKLEIKRTVAAPSVFIFPPSDEQLKSGTASVVCLLNNFYPREAKVQWKVDNALQSGNSQESVTEQDSKDSTYSLSSTLTLSKADYEKHKVYACEVTHQGLSSPVTKSFNRGECGGGGSGGGGSCDLPQTHSLGSRRTLMLLAQMRRISLFSCAKDRHDFGFPQEEFGNQFQKAETIPVLHEMIQQIFNLFSTKDSSAAWDETLLDKFYTELYQQLNDLEACVIQGVGVTETPLMKEDSILAVRKYFQRITLYLKEKKYSPCAWEVVRAEIMRSFSLSTNLQESLRSKEDKTHTCPPCPAPELLGGPSVFLFPPKPKDTLMISRTPEVTCVVVDVSHEDPEVKFNWYVDGVEVHNAKTKPREEQYNSTYRVVSVLTVLHQDWLNGKEYKCKVSNKALPAPIEKTISKAKGQPREPQVYTLPPSRDELTKNQVSLWCLVKGFYPSDIAVEWESNGQPENNYKTTPPVLDSDGSFFLYSKLTVDKSRWQQGNVFSCSVMHEALHNHYTQKSLSLSPGK

SEQ ID NO: 10 - protein, 621 aa, Artificial Sequence
  GC33(L)-(GGGGS)2-IFN 2bA145G-Fc2
DVVMTQSPLSLPVTPGEPASISCRSSQSLVHSNRNTYLHWYLQKPGQSPQLLIYKVSNRFSGVPDRFSGSGSGTDFTLKISRVEAEDVGVYYCSQNTHVPPTFGQGTKLEIKRTVAAPSVFIFPPSDEQLKSGTASVVCLLNNFYPREAKVQWKVDNALQSGNSQESVTEQDSKDSTYSLSSTLTLSKADYEKHKVYACEVTHQGLSSPVTKSFNRGECGGGGSGGGGSCDLPQTHSLGSRRTLMLLAQMRRISLFSCLKDRHDFGFPQEEFGNQFQKAETIPVLHEMIQQIFNLFSTKDSSAAWDETLLDKFYTELYQQLNDLEACVIQGVGVTETPLMKEDSILAVRKYFQRITLYLKEKKYSPCAWEVVRGEIMRSFSLSTNLQESLRSKEDKTHTCPPCPAPELLGGPSVFLFPPKPKDTLMISRTPEVTCVVVDVSHEDPEVKFNWYVDGVEVHNAKTKPREEQYNSTYRVVSVLTVLHQDWLNGKEYKCKVSNKALPAPIEKTISKAKGQPREPQVYTLPPSRDELTKNQVSLWCLVKGFYPSDIAVEWESNGQPENNYKTTPPVLDSDGSFFLYSKLTVDKSRWQQGNVFSCSVMHEALHNHYTQKSLSLSPGK

SEQ ID NO: 11 - protein, 621 aa, Artificial Sequence
  GC33(L)-(GGGGS)2-IFN 2bR149A-Fc2
DVVMTQSPLSLPVTPGEPASISCRSSQSLVHSNRNTYLHWYLQKPGQSPQLLIYKVSNRFSGVPDRFSGSGSGTDFTLKISRVEAEDVGVYYCSQNTHVPPTFGQGTKLEIKRTVAAPSVFIFPPSDEQLKSGTASVVCLLNNFYPREAKVQWKVDNALQSGNSQESVTEQDSKDSTYSLSSTLTLSKADYEKHKVYACEVTHQGLSSPVTKSFNRGECGGGGSGGGGSCDLPQTHSLGSRRTLMLLAQMRRISLFSCLKDRHDFGFPQEEFGNQFQKAETIPVLHEMIQQIFNLFSTKDSSAAWDETLLDKFYTELYQQLNDLEACVIQGVGVTETPLMKEDSILAVRKYFQRITLYLKEKKYSPCAWEVVRAEIMASFSLSTNLQESLRSKEDKTHTCPPCPAPELLGGPSVFLFPPKPKDTLMISRTPEVTCVVVDVSHEDPEVKFNWYVDGVEVHNAKTKPREEQYNSTYRVVSVLTVLHQDWLNGKEYKCKVSNKALPAPIEKTISKAKGQPREPQVYTLPPSRDELTKNQVSLWCLVKGFYPSDIAVEWESNGQPENNYKTTPPVLDSDGSFFLYSKLTVDKSRWQQGNVFSCSVMHEALHNHYTQKSLSLSPGK

SEQ ID NO: 12 - protein, 621 aa, Artificial Sequence
  GC33(L)-(GGGGS)2-IFN 2bS152A-Fc2
DVVMTQSPLSLPVTPGEPASISCRSSQSLVHSNRNTYLHWYLQKPGQSPQLLIYKVSNRFSGVPDRFSGSGSGTDFTLKISRVEAEDVGVYYCSQNTHVPPTFGQGTKLEIKRTVAAPSVFIFPPSDEQLKSGTASVVCLLNNFYPREAKVQWKVDNALQSGNSQESVTEQDSKDSTYSLSSTLTLSKADYEKHKVYACEVTHQGLSSPVTKSFNRGECGGGGSGGGGSCDLPQTHSLGSRRTLMLLAQMRRISLFSCLKDRHDFGFPQEEFGNQFQKAETIPVLHEMIQQIFNLFSTKDSSAAWDETLLDKFYTELYQQLNDLEACVIQGVGVTETPLMKEDSILAVRKYFQRITLYLKEKKYSPCAWEVVRAEIMRSFALSTNLQESLRSKEDKTHTCPPCPAPELLGGPSVFLFPPKPKDTLMISRTPEVTCVVVDVSHEDPEVKFNWYVDGVEVHNAKTKPREEQYNSTYRVVSVLTVLHQDWLNGKEYKCKVSNKALPAPIEKTISKAKGQPREPQVYTLPPSRDELTKNQVSLWCLVKGFYPSDIAVEWESNGQPENNYKTTPPVLDSDGSFFLYSKLTVDKSRWQQGNVFSCSVMHEALHNHYTQKSLSLSPGK

SEQ ID NO: 13 - protein, 631 aa, Artificial Sequence
  GC33(L)-(GGGGS)4-IFN 2bA145G-Fc2
DVVMTQSPLSLPVTPGEPASISCRSSQSLVHSNRNTYLHWYLQKPGQSPQLLIYKVSNRFSGVPDRFSGSGSGTDFTLKISRVEAEDVGVYYCSQNTHVPPTFGQGTKLEIKRTVAAPSVFIFPPSDEQLKSGTASVVCLLNNFYPREAKVQWKVDNALQSGNSQESVTEQDSKDSTYSLSSTLTLSKADYEKHKVYACEVTHQGLSSPVTKSFNRGECGGGGSGGGGSGGGGSGGGGSCDLPQTHSLGSRRTLMLLAQMRRISLFSCLKDRHDFGFPQEEFGNQFQKAETIPVLHEMIQQIFNLFSTKDSSAAWDETLLDKFYTELYQQLNDLEACVIQGVGVTETPLMKEDSILAVRKYFQRITLYLKEKKYSPCAWEVVRGEIMRSFSLSTNLQESLRSKEDKTHTCPPCPAPELLGGPSVFLFPPKPKDTLMISRTPEVTCVVVDVSHEDPEVKFNWYVDGVEVHNAKTKPREEQYNSTYRVVSVLTVLHQDWLNGKEYKCKVSNKALPAPIEKTISKAKGQPREPQVYTLPPSRDELTKNQVSLWCLVKGFYPSDIAVEWESNGQPENNYKTTPPVLDSDGSFFLYSKLTVDKSRWQQGNVFSCSVMHEALHNHYTQKSLSLSPGK

SEQ ID NO: 14 - protein, 631 aa, Artificial Sequence
  GC33(L)-(GGGGS)4-IFN 2bR149A-Fc2
DVVMTQSPLSLPVTPGEPASISCRSSQSLVHSNRNTYLHWYLQKPGQSPQLLIYKVSNRFSGVPDRFSGSGSGTDFTLKISRVEAEDVGVYYCSQNTHVPPTFGQGTKLEIKRTVAAPSVFIFPPSDEQLKSGTASVVCLLNNFYPREAKVQWKVDNALQSGNSQESVTEQDSKDSTYSLSSTLTLSKADYEKHKVYACEVTHQGLSSPVTKSFNRGECGGGGSGGGGSGGGGSGGGGSCDLPQTHSLGSRRTLMLLAQMRRISLFSCLKDRHDFGFPQEEFGNQFQKAETIPVLHEMIQQIFNLFSTKDSSAAWDETLLDKFYTELYQQLNDLEACVIQGVGVTETPLMKEDSILAVRKYFQRITLYLKEKKYSPCAWEVVRAEIMASFSLSTNLQESLRSKEDKTHTCPPCPAPELLGGPSVFLFPPKPKDTLMISRTPEVTCVVVDVSHEDPEVKFNWYVDGVEVHNAKTKPREEQYNSTYRVVSVLTVLHQDWLNGKEYKCKVSNKALPAPIEKTISKAKGQPREPQVYTLPPSRDELTKNQVSLWCLVKGFYPSDIAVEWESNGQPENNYKTTPPVLDSDGSFFLYSKLTVDKSRWQQGNVFSCSVMHEALHNHYTQKSLSLSPGK

SEQ ID NO: 15 - protein, 450 aa, Artificial Sequence
  Palivizumab(H)- Fc1
QVTLRESGPALVKPTQTLTLTCTFSGFSLSTSGMSVGWIRQPPGKALEWLADIWWDDKKDYNPSLKSRLTISKDTSKNQVVLKVTNMDPADTATYYCARSMITNWYFDVWGAGTTVTVSSASTKGPSVFPLAPSSKSTSGGTAALGCLVKDYFPEPVTVSWNSGALTSGVHTFPAVLQSSGLYSLSSVVTVPSSSLGTQTYICNVNHKPSNTKVDKKVEPKSCDKTHTCPPCPAPELLGGPSVFLFPPKPKDTLMISRTPEVTCVVVDVSHEDPEVKFNWYVDGVEVHNAKTKPREEQYNSTYRVVSVLTVLHQDWLNGKEYKCKVSNKALPAPIEKTISKAKGQPREPQVYTLPPSRDELTKNQVSLSCAVKGFYPSDIAVEWESNGQPENNYKTTPPVLDSDGSFFLVSKLTVDKSRWQQGNVFSCSVMHEALHNHYTQKSLSLSPGK

SEQ ID NO: 16 - protein, 615 aa, Artificial Sequence
  Palivizumab (L)-(GGGGS)2-IFN 2b-Fc2
DIQMTQSPSTLSASVGDRVTITCKCQLSVGYMHWYQQKPGKAPKLLIYDTSKLASGVPSRFSGSGSGTEFTLTISSLQPDDFATYYCFQGSGYPFTFGGGTKLEIKRTVAAPSVFIFPPSDEQLKSGTASVVCLLNNFYPREAKVQWKVDNALQSGNSQESVTEQDSKDSTYSLSSTLTLSKADYEKHKVYACEVTHQGLSSPVTKSFNRGECGGGGSGGGGSCDLPQTHSLGSRRTLMLLAQMRRISLFSCLKDRHDFGFPQEEFGNQFQKAETIPVLHEMIQQIFNLFSTKDSSAAWDETLLDKFYTELYQQLNDLEACVIQGVGVTETPLMKEDSILAVRKYFQRITLYLKEKKYSPCAWEVVRAEIMRSFSLSTNLQESLRSKEDKTHTCPPCPAPELLGGPSVFLFPPKPKDTLMISRTPEVTCVVVDVSHEDPEVKFNWYVDGVEVHNAKTKPREEQYNSTYRVVSVLTVLHQDWLNGKEYKCKVSNKALPAPIEKTISKAKGQPREPQVYTLPPSRDELTKNQVSLWCLVKGFYPSDIAVEWESNGQPENNYKTTPPVLDSDGSFFLYSKLTVDKSRWQQGNVFSCSVMHEALHNHYTQKSLSLSPGK

SEQ ID NO: 17 - protein, 415 aa, Artificial Sequence
  IFN- 2b-Fc1
MALTFALLVALLVLSCKSSCSVGCDLPQTHSLGSRRTLMLLAQMRRISLFSCLKDRHDFGFPQEEFGNQFQKAETIPVLHEMIQQIFNLFSTKDSSAAWDETLLDKFYTELYQQLNDLEACVIQGVGVTETPLMKEDSILAVRKYFQRITLYLKEKKYSPCAWEVVRAEIMRSFSLSTNLQESLRSKEDKTHTCPPCPAPELLGGPSVFLFPPKPKDTLMISRTPEVTCVVVDVSHEDPEVKFNWYVDGVEVHNAKTKPREEQYNSTYRVVSVLTVLHQDWLNGKEYKCKVSNKALPAPIEKTISKAKGQPREPQVYTLPPSRDELTKNQVSLTCLVKGFYPSDIAVEWESNGQPENNYKTTPPVLDSDGSFFLYSKLTVDKSRWQQGNVFSCSVMHEALHNHYTQKSLSLSPGK

SEQ ID NO: 18 - protein, 188 aa, Artificial Sequence
  IFN- 2b
MALTFALLVALLVLSCKSSCSVGCDLPQTHSLGSRRTLMLLAQMRRISLFSCLKDRHDFGFPQEEFGNQFQKAETIPVLHEMIQQIFNLFSTKDSSAAWDETLLDKFYTELYQQLNDLEACVIQGVGVTETPLMKEDSILAVRKYFQRITLYLKEKKYSPCAWEVVRAEIMRSFSLSTNLQESLRSKE

SEQ ID NO: 19 - protein, 445 aa, Artificial Sequence
  GC33(H)-Fc
QVQLVQSGAEVKKPGASVKVSCKASGYTFTDYEMHWVRQAPGQGLEWMGALDPKTGDTAYSQKFKGRVTLTADKSTSTAYMELSSLTSEDTAVYYCTRFYSYTYWGQGTLVTVSSASTKGPSVFPLAPSSKSTSGGTAALGCLVKDYFPEPVTVSWNSGALTSGVHTFPAVLQSSGLYSLSSVVTVPSSSLGTQTYICNVNHKPSNTKVDKKVEPKSCDKTHTCPPCPAPELLGGPSVFLFPPKPKDTLMISRTPEVTCVVVDVSHEDPEVKFNWYVDGVEVHNAKTKPREEQYNSTYRVVSVLTVLHQDWLNGKEYKCKVSNKALPAPIEKTISKAKGQPREPQVYTLPPSREEMTKNQVSLTCLVKGFYPSDIAVEWESNGQPENNYKTTPPVLDSDGSFFLYSKLTVDKSRWQQGNVFSCSVMHEALHNHYTQKSLSLSPGK

SEQ ID NO: 20 - protein, 219 aa, Artificial Sequence
  GC33(L)
DVVMTQSPLSLPVTPGEPASISCRSSQSLVHSNRNTYLHWYLQKPGQSPQLLIYKVSNRFSGVPDRFSGSGSGTDFTLKISRVEAEDVGVYYCSQNTHVPPTFGQGTKLEIKRTVAAPSVFIFPPSDEQLKSGTASVVCLLNNFYPREAKVQWKVDNALQSGNSQESVTEQDSKDSTYSLSSTLTLSKADYEKHKVYACEVTHQGLSSPVTKSFNRGEC

SEQ ID NO: 21 - protein, 448 aa, Artificial Sequence
  AtezolizumabH-Fc1
EVQLVESGGGLVQPGGSLRLSCAASGFTFSDSWIHWVRQAPGKGLEWVAWISPYGGSTYYADSVKGRFTISADTSKNTAYLQMNSLRAEDTAVYYCARRHWPGGFDYWGQGTLVTVSSASTKGPSVFPLAPSSKSTSGGTAALGCLVKDYFPEPVTVSWNSGALTSGVHTFPAVLQSSGLYSLSSVVTVPSSSLGTQTYICNVNHKPSNTKVDKKVEPKSCDKTHTCPPCPAPELLGGPSVFLFPPKPKDTLMISRTPEVTCVVVDVSHEDPEVKFNWYVDGVEVHNAKTKPREEQYASTYRVVSVLTVLHQDWLNGKEYKCKVSNKALPAPIEKTISKAKGQPREPQVYTLPPSREEMTKNQVSLTCLVKGFYPSDIAVEWESNGQPENNYKTTPPVLDSDGSFFLYSKLTVDKSRWQQGNVFSCSVMHEALHNHYTQKSLSLSPGK

SEQ ID NO: 22 - protein, 214 aa, Artificial Sequence
  AtezolizumabL
DIQMTQSPSSLSASVGDRVTITCRASQDVSTAVAWYQQKPGKAPKLLIYSASFLYSGVPSRFSGSGSGTDFTLTISSLQPEDFATYYCQQYLYHPATFGQGTKVEIKRTVAAPSVFIFPPSDEQLKSGTASVVCLLNNFYPREAKVQWKVDNALQSGNSQESVTEQDSKDSTYSLSSTLTLSKADYEKHKVYACEVTHQGLSSPVTKSFNRGEC

SEQ ID NO: 23 - protein, 448 aa, Artificial Sequence
  Atezolizumab (H)-Fc1
EVQLVESGGGLVQPGGSLRLSCAASGFTFSDSWIHWVRQAPGKGLEWVAWISPYGGSTYYADSVKGRFTISADTSKNTAYLQMNSLRAEDTAVYYCARRHWPGGFDYWGQGTLVTVSSASTKGPSVFPLAPSSKSTSGGTAALGCLVKDYFPEPVTVSWNSGALTSGVHTFPAVLQSSGLYSLSSVVTVPSSSLGTQTYICNVNHKPSNTKVDKKVEPKSCDKTHTCPPCPAPELLGGPSVFLFPPKPKDTLMISRTPEVTCVVVDVSHEDPEVKFNWYVDGVEVHNAKTKPREEQYNSTYRVVSVLTVLHQDWLNGKEYKCKVSNKALPAPIEKTISKAKGQPREPQVYTLPPSRDELTKNQVSLSCAVKGFYPSDIAVEWESNGQPENNYKTTPPVLDSDGSFFLVSKLTVDKSRWQQGNVFSCSVMHEALHNHYTQKSLSLSPGK

SEQ ID NO: 24 - protein, 611 aa, Artificial Sequence
  Atezolizumab (L)-(GGGGS)1-IFN 2b-Fc2
DIQMTQSPSSLSASVGDRVTITCRASQDVSTAVAWYQQKPGKAPKLLIYSASFLYSGVPSRFSGSGSGTDFTLTISSLQPEDFATYYCQQYLYHPATFGQGTKVEIKRTVAAPSVFIFPPSDEQLKSGTASVVCLLNNFYPREAKVQWKVDNALQSGNSQESVTEQDSKDSTYSLSSTLTLSKADYEKHKVYACEVTHQGLSSPVTKSFNRGECGGGGSCDLPQTHSLGSRRTLMLLAQMRRISLFSCLKDRHDFGFPQEEFGNQFQKAETIPVLHEMIQQIFNLFSTKDSSAAWDETLLDKFYTELYQQLNDLEACVIQGVGVTETPLMKEDSILAVRKYFQRITLYLKEKKYSPCAWEVVRAEIMRSFSLSTNLQESLRSKEDKTHTCPPCPAPELLGGPSVFLFPPKPKDTLMISRTPEVTCVVVDVSHEDPEVKFNWYVDGVEVHNAKTKPREEQYNSTYRVVSVLTVLHQDWLNGKEYKCKVSNKALPAPIEKTISKAKGQPREPQVYTLPPSRDELTKNQVSLWCLVKGFYPSDIAVEWESNGQPENNYKTTPPVLDSDGSFFLYSKLTVDKSRWQQGNVFSCSVMHEALHNHYTQKSLSLSPGK

SEQ ID NO: 25 - protein, 616 aa, Artificial Sequence
  Atezolizumab (L)-(GGGGS)2-IFN 2b-Fc2
DIQMTQSPSSLSASVGDRVTITCRASQDVSTAVAWYQQKPGKAPKLLIYSASFLYSGVPSRFSGSGSGTDFTLTISSLQPEDFATYYCQQYLYHPATFGQGTKVEIKRTVAAPSVFIFPPSDEQLKSGTASVVCLLNNFYPREAKVQWKVDNALQSGNSQESVTEQDSKDSTYSLSSTLTLSKADYEKHKVYACEVTHQGLSSPVTKSFNRGECGGGGSGGGGSCDLPQTHSLGSRRTLMLLAQMRRISLFSCLKDRHDFGFPQEEFGNQFQKAETIPVLHEMIQQIFNLFSTKDSSAAWDETLLDKFYTELYQQLNDLEACVIQGVGVTETPLMKEDSILAVRKYFQRITLYLKEKKYSPCAWEVVRAEIMRSFSLSTNLQESLRSKEDKTHTCPPCPAPELLGGPSVFLFPPKPKDTLMISRTPEVTCVVVDVSHEDPEVKFNWYVDGVEVHNAKTKPREEQYNSTYRVVSVLTVLHQDWLNGKEYKCKVSNKALPAPIEKTISKAKGQPREPQVYTLPPSRDELTKNQVSLWCLVKGFYPSDIAVEWESNGQPENNYKTTPPVLDSDGSFFLYSKLTVDKSRWQQGNVFSCSVMHEALHNHYTQKSLSLSPGK

SEQ ID NO: 26 - protein, 621 aa, Artificial Sequence
  Atezolizumab (L)-(GGGGS)3-IFN 2b-Fc2
DIQMTQSPSSLSASVGDRVTITCRASQDVSTAVAWYQQKPGKAPKLLIYSASFLYSGVPSRFSGSGSGTDFTLTISSLQPEDFATYYCQQYLYHPATFGQGTKVEIKRTVAAPSVFIFPPSDEQLKSGTASVVCLLNNFYPREAKVQWKVDNALQSGNSQESVTEQDSKDSTYSLSSTLTLSKADYEKHKVYACEVTHQGLSSPVTKSFNRGECGGGGSGGGGSGGGGSCDLPQTHSLGSRRTLMLLAQMRRISLFSCLKDRHDFGFPQEEFGNQFQKAETIPVLHEMIQQIFNLFSTKDSSAAWDETLLDKFYTELYQQLNDLEACVIQGVGVTETPLMKEDSILAVRKYFQRITLYLKEKKYSPCAWEVVRAEIMRSFSLSTNLQESLRSKEDKTHTCPPCPAPELLGGPSVFLFPPKPKDTLMISRTPEVTCVVVDVSHEDPEVKFNWYVDGVEVHNAKTKPREEQYNSTYRVVSVLTVLHQDWLNGKEYKCKVSNKALPAPIEKTISKAKGQPREPQVYTLPPSRDELTKNQVSLWCLVKGFYPSDIAVEWESNGQPENNYKTTPPVLDSDGSFFLYSKLTVDKSRWQQGNVFSCSVMHEALHNHYTQKSLSLSPGK

SEQ ID NO: 27 - protein, 446 aa, Artificial Sequence
  Edrecolomab (H)-Fc1
QVQLQQSGAELVRPGTSVKVSCKASGYAFTNYLIEWVKQRPGQGLEWIGVINPGSGGTNYNEKFKGKATLTADKSSSTAYMQLSSLTSDDSAVYFCARDGPWFAYWGQGTLVTVSAASTKGPSVFPLAPSSKSTSGGTAALGCLVKDYFPEPVTVSWNSGALTSGVHTFPAVLQSSGLYSLSSVVTVPSSSLGTQTYICNVNHKPSNTKVDKKVEPKSCDKTHTCPPCPAPELLGGPSVFLFPPKPKDTLMISRTPEVTCVVVDVSHEDPEVKFNWYVDGVEVHNAKTKPREEQYNSTYRVVSVLTVLHQDWLNGKEYKCKVSNKALPAPIEKTISKAKGQPREPQVYTLPPSRDELTKNQVSLSCAVKGFYPSDIAVEWESNGQPENNYKTTPPVLDSDGSFFLVSKLTVDKSRWQQGNVFSCSVMHEALHNHYTQKSLSLSPGK

SEQ ID NO: 28 - protein, 583 aa, Artificial Sequence
  Edrecolomab (L)-(GGGGS)5- SIRPD1-Fc2
NIVMTQSPKSMSMSVGERVTLTCKASENVVTYVSWYQQKPEQSPKLLIYGASNRYTGVPDRFTGSGSATDFTLTISSVQAEDLADYHCGQGYSYPYTFGGGTKLEIKRTVAAPSVFIFPPSDEQLKSGTASVVCLLNNFYPREAKVQWKVDNALQSGNSQESVTEQDSKDSTYSLSSTLTLSKADYEKHKVYACEVTHQGLSSPVTKSFNRGECGGGGSGGGGSGGGGSGGGGSGGGGSEEELQVIQPDKSVSVAAGESAILHCTVTSLIPVGPIQWFRGAGPARELIYNQKEGHFPRVTTVSESTKRENMDFSISISAITPADAGTYYCVKFRKGSPDTEFKSGAGTELSVRAKPDKTHTCPPCPAPELLGGPSVFLFPPKPKDTLMISRTPEVTCVVVDVSHEDPEVKFNWYVDGVEVHNAKTKPREEQYNSTYRVVSVLTVLHQDWLNGKEYKCKVSNKALPAPIEKTISKAKGQPREPQVYTLPPSRDELTKNQVSLWCLVKGFYPSDIAVEWESNGQPENNYKTTPPVLDSDGSFFLYSKLTVDKSRWQQGNVFSCSVMHEALHNHYTQKSLSLSPGK

SEQ ID NO: 29 - protein, 448 aa, Artificial Sequence
  SWA11(H)-Fc1
DVHLQESGPDLVKPSQSLSLTCTVTGYSITSGYTWHWIRQFPGNTVEWMGYIQYTGSTRYNPALRGRLSISRDTSKNQFFLQLISVTTADTGTYFCARGTTASFDYWGQGTTLTVASAASTKGPSVFPLAPSSKSTSGGTAALGCLVKDYFPEPVTVSWNSGALTSGVHTFPAVLQSSGLYSLSSVVTVPSSSLGTQTYICNVNHKPSNTKVDKRVEPKSCDKTHTCPPCPAPELLGGPSVFLFPPKPKDTLMISRTPEVTCVVVDVSHEDPEVKFNWYVDGVEVHNAKTKPREEQYNSTYRVVSVLTVLHQDWLNGKEYKCKVSNKALPAPIEKTISKAKGQPREPQVYTLPPSRDELTKNQVSLSCAVKGFYPSDIAVEWESNGQPENNYKTTPPVLDSDGSFFLVSKLTVDKSRWQQGNVFSCSVMHEALHNHYTQKSLSLSPGK

SEQ ID NO: 30 - protein, 574 aa, Artificial Sequence
  SWA11(L)-(GGGGS)2- SIRPD1-Fc2
DIVMSQSPSSLNVSVGEKVTMRCRSSQSLLYSSDQKNYLTWYQQKPGQSPKLLISWASTRASGVPDRFTGSGSGTDFTLTISSVKAEDLGVYYCQQYFIYPLTFGVGTKLGLKRTVAAPSVFIFPPSDEQLKSGTASVVCLLNNFYPREAKVQWKVDNALQSGNSQESVTEQDSKDSTYSLSSTLTLSKADYEKHKVYACEVTHQGLSSPVTKSFNRGECGGGGSGGGGSEEELQVIQPDKSVSVAAGESAILHCTVTSLIPVGPIQWFRGAGPARELIYNQKEGHFPRVTTVSESTKRENMDFSISISAITPADAGTYYCVKFRKGSPDTEFKSGAGTELSVRAKPDKTHTCPPCPAPELLGGPSVFLFPPKPKDTLMISRTPEVTCVVVDVSHEDPEVKFNWYVDGVEVHNAKTKPREEQYNSTYRVVSVLTVLHQDWLNGKEYKCKVSNKALPAPIEKTISKAKGQPREPQVYTLPPSRDELTKNQVSLWCLVKGFYPSDIAVEWESNGQPENNYKTTPPVLDSDGSFFLYSKLTVDKSRWQQGNVFSCSVMHEALHNHYTQKSLSLSPGK

SEQ ID NO: 31 - protein, 444 aa, Artificial Sequence
  Mezagitamab(L)-Fc1
QSVLTQPPSASGTPGQRVTISCSGSSSNIGDNYVSWYQQLPGTAPKLLIYRDSQRPSGVPDRFSGSKSGTSASLAISGLRSEDEADYYCQSYDSSLSGSVFGGGTKLTVLGQPKANPTVTLFPPSSEELQANKATLVCLISDFYPGAVTVAWKADGSPVKAGVETTKPSKQSNNKYAASSYLSLTPEQWKSHRSYSCQVTHEGSTVEKTVAPTECSCDKTHTCPPCPAPELLGGPSVFLFPPKPKDTLMISRTPEVTCVVVDVSHEDPEVKFNWYVDGVEVHNAKTKPREEQYNSTYRVVSVLTVLHQDWLNGKEYKCKVSNKALPAPIEKTISKAKGQPREPQVYTLPPSRDELTKNQVSLSCAVKGFYPSDIAVEWESNGQPENNYKTTPPVLDSDGSFFLVSKLTVDKSRWQQGNVFSCSVMHEALHNHYTQKSLSLSPGK

SEQ ID NO: 32 - protein, 643 aa, Artificial Sequence
  Mezagitamab (H)-(GGGGS)5-IFN2b-Fc2
EVQLLESGGGLVQPGGSLRLSCAASGFTFDDYGMSWVRQAPGKGLEWVSDISWNGGKTHYVDSVKGQFTISRDNSKNTLYLQMNSLRAEDTAVYYCARGSLFHDSSGFYFGHWGQGTLVTVSSASTKGPSVFPLAPSSKSTSGGTAALGCLVKDYFPEPVTVSWNSGALTSGVHTFPAVLQSSGLYSLSSVVTVPSSSLGTQTYICNVNHKPSNTKVDKKVEPKSCGGGGSGGGGSGGGGSGGGGSGGGGSCDLPQTHSLGSRRTLMLLAQMRRISLFSCLKDRHDFGFPQEEFGNQFQKAETIPVLHEMIQQIFNLFSTKDSSAAWDETLLDKFYTELYQQLNDLEACVIQGVGVTETPLMKEDSILAVRKYFQRITLYLKEKKYSPCAWEVVRAEIMRSFSLSTNLQESLRSKEDKTHTCPPCPAPELLGGPSVFLFPPKPKDTLMISRTPEVTCVVVDVSHEDPEVKFNWYVDGVEVHNAKTKPREEQYNSTYRVVSVLTVLHQDWLNGKEYKCKVSNKALPAPIEKTISKAKGQPREPQVYTLPPSRDELTKNQVSLWCLVKGFYPSDIAVEWESNGQPENNYKTTPPVLDSDGSFFLYSKLTVDKSRWQQGNVFSCSVMHEALHNHYTQKSLSLSPGK

SEQ ID NO: 33 - protein, 450 aa, Artificial Sequence
  Felzartamab(H)-Fc2
QVQLVESGGGLVQPGGSLRLSCAASGFTFSSYYMNWVRQAPGKGLEWVSGISGDPSNTYYADSVKGRFTISRDNSKNTLYLQMNSLRAEDTAVYYCARDLPLVYTGFAYWGQGTLVTVSSASTKGPSVFPLAPSSKSTSGGTAALGCLVKDYFPEPVTVSWNSGALTSGVHTFPAVLQSSGLYSLSSVVTVPSSSLGTQTYICNVNHKPSNTKVDKKVEPKSCDKTHTCPPCPAPELLGGPSVFLFPPKPKDTLMISRTPEVTCVVVDVSHEDPEVKFNWYVDGVEVHNAKTKPREEQYNSTYRVVSVLTVLHQDWLNGKEYKCKVSNKALPAPIEKTISKAKGQPREPQVYTLPPSRDELTKNQVSLWCLVKGFYPSDIAVEWESNGQPENNYKTTPPVLDSDGSFFLYSKLTVDKSRWQQGNVFSCSVMHEALHNHYTQKSLSLSPGK

SEQ ID NO: 34 - protein, 582 aa, Artificial Sequence
  Felzartamab(L)-(GGGGS)5- SIRPD1-Fc1
DIELTQPPSVSVAPGQTARISCSGDNLRHYYVYWYQQKPGQAPVLVIYGDSKRPSGIPERFSGSNSGNTATLTISGTQAEDEADYYCQTYTGGASLVFGGGTKLTVLGQPKAAPSVTLFPPSSEELQANKATLVCLISDFYPGAVTVAWKADSSPVKAGVETTTPSKQSNNKYAASSYLSLTPEQWKSHRSYSCQVTHEGSTVEKTVAPTECSGGGGSGGGGSGGGGSGGGGSGGGGSEEELQVIQPDKSVSVAAGESAILHCTVTSLIPVGPIQWFRGAGPARELIYNQKEGHFPRVTTVSESTKRENMDFSISISAITPADAGTYYCVKFRKGSPDTEFKSGAGTELSVRAKPDKTHTCPPCPAPELLGGPSVFLFPPKPKDTLMISRTPEVTCVVVDVSHEDPEVKFNWYVDGVEVHNAKTKPREEQYNSTYRVVSVLTVLHQDWLNGKEYKCKVSNKALPAPIEKTISKAKGQPREPQVYTLPPSRDELTKNQVSLSCAVKGFYPSDIAVEWESNGQPENNYKTTPPVLDSDGSFFLVSKLTVDKSRWQQGNVFSCSVMHEALHNHYTQKSLSLSPGK

SEQ ID NO: 35 - protein, 456 aa, Artificial Sequence
  Tiragolumab(H)-Fc1
EVQLQQSGPGLVKPSQTLSLTCAISGDSVSSNSAAWNWIRQSPSRGLEWLGKTYYRFKWYSDYAVSVKGRITINPDTSKNQFSLQLNSVTPEDTAVFYCTRESTTYDLLAGPFDYWGQGTLVTVSSASTKGPSVFPLAPSSKSTSGGTAALGCLVKDYFPEPVTVSWNSGALTSGVHTFPAVLQSSGLYSLSSVVTVPSSSLGTQTYICNVNHKPSNTKVDKKVEPKSCDKTHTCPPCPAPELLGGPSVFLFPPKPKDTLMISRTPEVTCVVVDVSHEDPEVKFNWYVDGVEVHNAKTKPREEQYNSTYRVVSVLTVLHQDWLNGKEYKCKVSNKALPAPIEKTISKAKGQPREPQVYTLPPSREEMTKNQVSLSCAVKGFYPSDIAVEWESNGQPENNYKTTPPVLDSDGSFFLVSKLTVDKSRWQQGNVFSCSVMHEALHNHYTQKSLSLSPGK

SEQ ID NO: 36 - protein, 664 aa, Artificial Sequence
  Tiragolumab (L)-(GGGGS)4-IL12A-Fc2
DIVMTQSPDSLAVSLGERATINCKSSQTVLYSSNNKKYLAWYQQKPGQPPNLLIYWASTRESGVPDRFSGSGSGTDFTLTISSLQAEDVAVYYCQQYYSTPFTFGPGTKVEIKRTVAAPSVFIFPPSDEQLKSGTASVVCLLNNFYPREAKVQWKVDNALQSGNSQESVTEQDSKDSTYSLSSTLTLSKADYEKHKVYACEVTHQGLSSPVTKSFNRGECGGGGSGGGGSGGGGSGGGGSRNLPVATPDPGMFPCLHHSQNLLRAVSNMLQKARQTLEFYPCTSEEIDHEDITKDKTSTVEACLPLELTKNESCLNSRETSFITNGSCLASRKTSFMMALCLSSIYEDLKMYQVEFKTMNAKLLMDPKRQIFLDQNMLAVIDELMQALNFNSETVPQKSSLEEPDFYKTKIKLCILLHAFRIRAVTIDRVMSYLNASDKTHTCPPCPAPELLGGPSVFLFPPKPKDTLMISRTPEVTCVVVDVSHEDPEVKFNWYVDGVEVHNAKTKPREEQYNSTYRVVSVLTVLHQDWLNGKEYKCKVSNKALPAPIEKTISKAKGQPREPQVYTLPPSREEMTKNQVSLWCLVKGFYPSDIAVEWESNGQPENNYKTTPPVLDSDGSFFLYSKLTVDKSRWQQGNVFSCSVMHEALHNHYTQKSLSLSPGK

SEQ ID NO: 37 - protein, 457 aa, Artificial Sequence
  Galiximab(H)-Fc1
QVQLQESGPGLVKPSETLSLTCAVSGGSISGGYGWGWIRQPPGKGLEWIGSFYSSSGNTYYNPSLKSQVTISTDTSKNQFSLKLNSMTAADTAVYYCVRDRLFSVVGMVYNNWFDVWGPGVLVTVSSASTKGPSVFPLAPSSKSTSGGTAALGCLVKDYFPEPVTVSWNSGALTSGVHTFPAVLQSSGLYSLSSVVTVPSSSLGTQTYICNVNHKPSNTKVDKKVEPKSCDKTHTCPPCPAPEAAGGPSVFLFPPKPKDTLMISRTPEVTCVVVDVSHEDPEVKFNWYVDGVEVHNAKTKPREEQYNSTYRVVSVLTVLHQDWLNGKEYKCKVSNKALPAPIEKTISKAKGQPREPQVYTLPPSRDELTKNQVSLSCAVKGFYPSDIAVEWESNGQPENNYKTTPPVLDSDGSFFLVSKLTVDKSRWQQGNVFSCSVMHEALHNHYTQKSLSLSPGK

SEQ ID NO: 38 - protein, 634 aa, Artificial Sequence
  Galiximab(L)- (GGGGS)5-IL10M-Fc2
ESVLTQPPSVSGAPGQKVTISCTGSTSNIGGYDLHWYQQLPGTAPKLLIYDINKRPSGISDRFSGSKSGTAASLAITGLQTEDEADYYCQSYDSSLNAQVFGGGTRLTVLGQPKAAPSVTLFPPSSEELQANKATLVCLISDFYPGAVTVAWKADSSPVKAGVETTTPSKQSNNKYAASSYLSLTPEQWKSHRSYSCQVTHEGSTVEKTVAPTECSGGGGSGGGGSGGGGSGGGGSGGGGSSPGQGTQSENSCTHFPGNLPNMLRDLRDAFSRVKTFFQMKDQLDNLLLKESLLEDFKGYLGCQALSEMIQFYLEEVMPQAENQDPDIKAHVNSLGENLKTLRLRLRRCHRFLPCENGGGSGGKSKAVEQVKNAFNKLQEKGIYKAMSEFDIFINYIEAYMTMKIRNDKTHTCPPCPAPEAAGGPSVFLFPPKPKDTLMISRTPEVTCVVVDVSHEDPEVKFNWYVDGVEVHNAKTKPREEQYNSTYRVVSVLTVLHQDWLNGKEYKCKVSNKALPAPIEKTISKAKGQPREPQVYTLPPSRDELTKNQVSLWCLVKGFYPSDIAVEWESNGQPENNYKTTPPVLDSDGSFFLYSKLTVDKSRWQQGNVFSCSVMHEALHNHYTQKSLSLSPGK

SEQ ID NO: 39 - protein, 443 aa, Artificial Sequence
  Nivolumab(H)-Fc1
QVQLVESGGGVVQPGRSLRLDCKASGITFSNSGMHWVRQAPGKGLEWVAVIWYDGSKRYYADSVKGRFTISRDNSKNTLFLQMNSLRAEDTAVYYCATNDDYWGQGTLVTVSSASTKGPSVFPLAPSSKSTSGGTAALGCLVKDYFPEPVTVSWNSGALTSGVHTFPAVLQSSGLYSLSSVVTVPSSSLGTQTYICNVNHKPSNTKVDKKVEPKSCDKTHTCPPCPAPEAAGGPSVFLFPPKPKDTLMISRTPEVTCVVVDVSHEDPEVKFNWYVDGVEVHNAKTKPREEQYNSTYRVVSVLTVLHQDWLNGKEYKCKVSNKALGAPIEKTISKAKGQPREPQVYTLPPSRDELTKNQVSLSCAVKGFYPSDIAVEWESNGQPENNYKTTPPVLDSDGSFFLVSKLTVDKSRWQQGNVFSCSVMHEALHNHYTQKSLSLSPGK

SEQ ID NO: 40 - protein, 675 aa, Artificial Sequence
  Nivolumab(L)-(GGGGS)5-IL15-(GGGGS)5- IL15RSUSHI-Fc2
EIVLTQSPATLSLSPGERATLSCRASQSVSSYLAWYQQKPGQAPRLLIYDASNRATGIPARFSGSGSGTDFTLTISSLEPEDFAVYYCQQSSNWPRTFGQGTKVEIKRTVAAPSVFIFPPSDEQLKSGTASVVCLLNNFYPREAKVQWKVDNALQSGNSQESVTEQDSKDSTYSLSSTLTLSKADYEKHKVYACEVTHQGLSSPVTKSFNRGECGGGGSGGGGSGGGGSGGGGSGGGGSNWVNVISDLKKIEDLIQSMHIDATLYTESDVHPSCKVTAMKCFLLELQVISLESGDASIHDTVENLIILANNSLSSNGNVTESGCKECEELEEKNIKEFLQSFVHIVQMFINTSGGGGSGGGGSGGGGSGGGGSGGGGSITCPPPMSVEHADIWVKSYSLYSRERYICNSGFKRKAGTSSLTECVLNKATNVAHWTTPSLKCIREPKSSDKTHTCPPCPAPEAAGGPSVFLFPPKPKDTLMISRTPEVTCVVVDVSHEDPEVKFNWYVDGVEVHNAKTKPREEQYNSTYRVVSVLTVLHQDWLNGKEYKCKVSNKALGAPIEKTISKAKGQPREPQVYTLPPSRDELTKNQVSLWCLVKGFYPSDIAVEWESNGQPENNYKTTPPVLDSDGSFFLYSKLTVDKSRWQQGNVFSCSVMHEALHNHYTQKSLSLSPGK

SEQ ID NO: 41 - protein, 675 aa, Artificial Sequence
  Nivolumab(L)-(GGGGS)5-IL15RSUSHI-(GGGGS)5-IL15-Fc2
EIVLTQSPATLSLSPGERATLSCRASQSVSSYLAWYQQKPGQAPRLLIYDASNRATGIPARFSGSGSGTDFTLTISSLEPEDFAVYYCQQSSNWPRTFGQGTKVEIKRTVAAPSVFIFPPSDEQLKSGTASVVCLLNNFYPREAKVQWKVDNALQSGNSQESVTEQDSKDSTYSLSSTLTLSKADYEKHKVYACEVTHQGLSSPVTKSFNRGECGGGGSGGGGSGGGGSGGGGSGGGGSITCPPPMSVEHADIWVKSYSLYSRERYICNSGFKRKAGTSSLTECVLNKATNVAHWTTPSLKCIRGGGGSGGGGSGGGGSGGGGSGGGGSNWVNVISDLKKIEDLIQSMHIDATLYTESDVHPSCKVTAMKCFLLELQVISLESGDASIHDTVENLIILANNSLSSNGNVTESGCKECEELEEKNIKEFLQSFVHIVQMFINTSEPKSSDKTHTCPPCPAPEAAGGPSVFLFPPKPKDTLMISRTPEVTCVVVDVSHEDPEVKFNWYVDGVEVHNAKTKPREEQYNSTYRVVSVLTVLHQDWLNGKEYKCKVSNKALGAPIEKTISKAKGQPREPQVYTLPPSRDELTKNQVSLWCLVKGFYPSDIAVEWESNGQPENNYKTTPPVLDSDGSFFLYSKLTVDKSRWQQGNVFSCSVMHEALHNHYTQKSLSLSPGK

SEQ ID NO: 42 - protein, 631 aa, Artificial Sequence
  Palivizumab (L)- (GGGGS)5-IL10M-Fc2
DIQMTQSPSTLSASVGDRVTITCKCQLSVGYMHWYQQKPGKAPKLLIYDTSKLASGVPSRFSGSGSGTEFTLTISSLQPDDFATYYCFQGSGYPFTFGGGTKLEIKRTVAAPSVFIFPPSDEQLKSGTASVVCLLNNFYPREAKVQWKVDNALQSGNSQESVTEQDSKDSTYSLSSTLTLSKADYEKHKVYACEVTHQGLSSPVTKSFNRGECGGGGSGGGGSGGGGSGGGGSGGGGSSPGQGTQSENSCTHFPGNLPNMLRDLRDAFSRVKTFFQMKDQLDNLLLKESLLEDFKGYLGCQALSEMIQFYLEEVMPQAENQDPDIKAHVNSLGENLKTLRLRLRRCHRFLPCENGGGSGGKSKAVEQVKNAFNKLQEKGIYKAMSEFDIFINYIEAYMTMKIRNDKTHTCPPCPAPEAAGGPSVFLFPPKPKDTLMISRTPEVTCVVVDVSHEDPEVKFNWYVDGVEVHNAKTKPREEQYNSTYRVVSVLTVLHQDWLNGKEYKCKVSNKALPAPIEKTISKAKGQPREPQVYTLPPSRDELTKNQVSLWCLVKGFYPSDIAVEWESNGQPENNYKTTPPVLDSDGSFFLYSKLTVDKSRWQQGNVFSCSVMHEALHNHYTQKSLSLSPGK

SEQ ID NO: 43 - protein, 674 aa, Artificial Sequence
  Palivizumab(L)-(GGGGS)5-IL15-(GGGGS)5- IL15RSUSHI-Fc2
DIQMTQSPSTLSASVGDRVTITCKCQLSVGYMHWYQQKPGKAPKLLIYDTSKLASGVPSRFSGSGSGTEFTLTISSLQPDDFATYYCFQGSGYPFTFGGGTKLEIKRTVAAPSVFIFPPSDEQLKSGTASVVCLLNNFYPREAKVQWKVDNALQSGNSQESVTEQDSKDSTYSLSSTLTLSKADYEKHKVYACEVTHQGLSSPVTKSFNRGECGGGGSGGGGSGGGGSGGGGSGGGGSNWVNVISDLKKIEDLIQSMHIDATLYTESDVHPSCKVTAMKCFLLELQVISLESGDASIHDTVENLIILANNSLSSNGNVTESGCKECEELEEKNIKEFLQSFVHIVQMFINTSGGGGSGGGGSGGGGSGGGGSGGGGSITCPPPMSVEHADIWVKSYSLYSRERYICNSGFKRKAGTSSLTECVLNKATNVAHWTTPSLKCIREPKSSDKTHTCPPCPAPEAAGGPSVFLFPPKPKDTLMISRTPEVTCVVVDVSHEDPEVKFNWYVDGVEVHNAKTKPREEQYNSTYRVVSVLTVLHQDWLNGKEYKCKVSNKALGAPIEKTISKAKGQPREPQVYTLPPSRDELTKNQVSLWCLVKGFYPSDIAVEWESNGQPENNYKTTPPVLDSDGSFFLYSKLTVDKSRWQQGNVFSCSVMHEALHNHYTQKSLSLSPGK

SEQ ID NO: 44 - protein, 674 aa, Artificial Sequence
  Palivizumab (L)-(GGGGS)5-IL15RSUSHI-(GGGGS)5-IL15-Fc2
DIQMTQSPSTLSASVGDRVTITCKCQLSVGYMHWYQQKPGKAPKLLIYDTSKLASGVPSRFSGSGSGTEFTLTISSLQPDDFATYYCFQGSGYPFTFGGGTKLEIKRTVAAPSVFIFPPSDEQLKSGTASVVCLLNNFYPREAKVQWKVDNALQSGNSQESVTEQDSKDSTYSLSSTLTLSKADYEKHKVYACEVTHQGLSSPVTKSFNRGECGGGGSGGGGSGGGGSGGGGSGGGGSITCPPPMSVEHADIWVKSYSLYSRERYICNSGFKRKAGTSSLTECVLNKATNVAHWTTPSLKCIRGGGGSGGGGSGGGGSGGGGSGGGGSNWVNVISDLKKIEDLIQSMHIDATLYTESDVHPSCKVTAMKCFLLELQVISLESGDASIHDTVENLIILANNSLSSNGNVTESGCKECEELEEKNIKEFLQSFVHIVQMFINTSEPKSSDKTHTCPPCPAPEAAGGPSVFLFPPKPKDTLMISRTPEVTCVVVDVSHEDPEVKFNWYVDGVEVHNAKTKPREEQYNSTYRVVSVLTVLHQDWLNGKEYKCKVSNKALGAPIEKTISKAKGQPREPQVYTLPPSRDELTKNQVSLWCLVKGFYPSDIAVEWESNGQPENNYKTTPPVLDSDGSFFLYSKLTVDKSRWQQGNVFSCSVMHEALHNHYTQKSLSLSPGK

SEQ ID NO: 45 - protein, 450 aa, Artificial Sequence
  Felzartamab(H)-Fc
QVQLVESGGGLVQPGGSLRLSCAASGFTFSSYYMNWVRQAPGKGLEWVSGISGDPSNTYYADSVKGRFTISRDNSKNTLYLQMNSLRAEDTAVYYCARDLPLVYTGFAYWGQGTLVTVSSASTKGPSVFPLAPSSKSTSGGTAALGCLVKDYFPEPVTVSWNSGALTSGVHTFPAVLQSSGLYSLSSVVTVPSSSLGTQTYICNVNHKPSNTKVDKRVEPKSCDKTHTCPPCPAPELLGGPSVFLFPPKPKDTLMISRTPEVTCVVVDVSHEDPEVKFNWYVDGVEVHNAKTKPREEQYNSTYRVVSVLTVLHQDWLNGKEYKCKVSNKALPAPIEKTISKAKGQPREPQVYTLPPSREEMTKNQVSLTCLVKGFYPSDIAVEWESNGQPENNYKTTPPVLDSDGSFFLYSKLTVDKSRWQQGNVFSCSVMHEALHNHYTQKSLSLSPGK

SEQ ID NO: 46 - protein, 213 aa, Artificial Sequence
  Felzartamab(L)
DIELTQPPSVSVAPGQTARISCSGDNLRHYYVYWYQQKPGQAPVLVIYGDSKRPSGIPERFSGSNSGNTATLTISGTQAEDEADYYCQTYTGGASLVFGGGTKLTVLGQPKAAPSVTLFPPSSEELQANKATLVCLISDFYPGAVTVAWKADSSPVKAGVETTTPSKQSNNKYAASSYLSLTPEQWKSHRSYSCQVTHEGSTVEKTVAPTECS

SEQ ID NO: 47 - protein, 393 aa, Artificial Sequence
  IL10M-Fc
SPGQGTQSENSCTHFPGNLPNMLRDLRDAFSRVKTFFQMKDQLDNLLLKESLLEDFKGYLGCQALSEMIQFYLEEVMPQAENQDPDIKAHVNSLGENLKTLRLRLRRCHRFLPCENGGGSGGKSKAVEQVKNAFNKLQEKGIYKAMSEFDIFINYIEAYMTMKIRNDKTHTCPPCPAPEAAGGPSVFLFPPKPKDTLMISRTPEVTCVVVDVSHEDPEVKFNWYVDGVEVHNAKTKPREEQYNSTYRVVSVLTVLHQDWLNGKEYKCKVSNKALPAPIEKTISKAKGQPREPQVYTLPPSRDELTKNQVSLTCLVKGFYPSDIAVEWESNGQPENNYKTTPPVLDSDGSFFLYSKLTVDKSRWQQGNVFSCSVMHEALHNHYTQKSLSLSPGK

SEQ ID NO: 48 - protein, 322 aa, Artificial Sequence
  IL12B
MRAWIFFLLCLAGRALAWELKKDVYVVELDWYPDAPGEMVVLTCDTPEEDGITWTLDQSSEVLGSGKTLTIQVKEFGDAGQYTCHKGGEVLSHSLLLLHKKEDGIWSTDILKDQKEPKNKTFLRCEAKNYSGRFTCWWLTTISTDLTFSVKSSRGSSDPQGVTCGAATLSAERVRGDNKEYEYSVECQEDSACPAAEESLPIEVMVDAVHKLKYENYTSSFFIRDIIKPDPPKNLQLKPLKNSRQVEVSWEYPDTWSTPHSYFSLTFCVQVQGKSKREKKDRVFTDKTSATVICRKNASISVRAQDRYYSSSWSEWASVPCS

SEQ ID NO: 49 - protein, 17 aa, Artificial Sequence
  Signal peptide
MRAWIFFLLCLAGRALA

SEQ ID NO: 50 - protein, 117 aa, Artificial Sequence
  SIRPD1
EEELQVIQPDKSVSVAAGESAILHCTVTSLIPVGPIQWFRGAGPARELIYNQKEGHFPRVTTVSESTKRENMDFSISISAITPADAGTYYCVKFRKGSPDTEFKSGAGTELSVRAKP

SEQ ID NO: 51 - protein, 197 aa, Artificial Sequence
  IL-12A
RNLPVATPDPGMFPCLHHSQNLLRAVSNMLQKARQTLEFYPCTSEEIDHEDITKDKTSTVEACLPLELTKNESCLNSRETSFITNGSCLASRKTSFMMALCLSSIYEDLKMYQVEFKTMNAKLLMDPKRQIFLDQNMLAVIDELMQALNFNSETVPQKSSLEEPDFYKTKIKLCILLHAFRIRAVTIDRVMSYLNAS

SEQ ID NO: 52 - protein, 166 aa, Artificial Sequence
  IL-10M
SPGQGTQSENSCTHFPGNLPNMLRDLRDAFSRVKTFFQMKDQLDNLLLKESLLEDFKGYLGCQALSEMIQFYLEEVMPQAENQDPDIKAHVNSLGENLKTLRLRLRRCHRFLPCENGGGSGGKSKAVEQVKNAFNKLQEKGIYKAMSEFDIFINYIEAYMTMKIRN

SEQ ID NO: 53 - protein, 114 aa, Artificial Sequence
  IL-15
NWVNVISDLKKIEDLIQSMHIDATLYTESDVHPSCKVTAMKCFLLELQVISLESGDASIHDTVENLIILANNSLSSNGNVTESGCKECEELEEKNIKEFLQSFVHIVQMFINTS

SEQ ID NO: 54 - protein, 65 aa, Artificial Sequence
  IL-15RSUSHI
ITCPPPMSVEHADIWVKSYSLYSRERYICNSGFKRKAGTSSLTECVLNKATNVAHWTTPSLKCIR

SEQ ID NO: 55 - protein, 166 aa, Artificial Sequence
  IFN
MSYNLLGFLQRSSNFQCQKLLWQLNGRLEYCLKDRMNFDIPEEIKQLQQFQKEDAALTIYEMLQNIFAIFRQDSSSTGWNETIVENLLANVYHQINHLKTVLEEKLEKEDFTRGKLMSSLHLKRYYGRILHYLKAKEYSHCAWTIVRVEILRNFYFINRLTGYLRN

SEQ ID NO: 56 - protein, 449 aa, Artificial Sequence
  Panitumumab (H)-Fc1
QVQLQESGPGLVKPSETLSLTCTVSGGSVSSGDYYWTWIRQSPGKGLEWIGHIYYSGNTNYNPSLKSRLTISIDTSKTQFSLKLSSVTAADTAIYYCVRDRVTGAFDIWGQGTMVTVSSASTKGPSVFPLAPSSKSTSGGTAALGCLVKDYFPEPVTVSWNSGALTSGVHTFPAVLQSSGLYSLSSVVTVPSSSLGTQTYICNVNHKPSNTKVDKKVEPKSCDKTHTCPPCPAPELLGGPSVFLFPPKPKDTLMISRTPEVTCVVVDVSHEDPEVKFNWYVDGVEVHNAKTKPREEQYNSTYRVVSVLTVLHQDWLNGKEYKCKVSNKALPAPIEKTISKAKGQPREPQVYTLPPSRDELTKNQVSLSCAVKGFYPSDIAVEWESNGQPENNYKTTPPVLDSDGSFFLVSKLTVDKSRWQQGNVFSCSVMHEALHNHYTQKSLSLSPGK

SEQ ID NO: 57 - protein, 573 aa, Artificial Sequence
  Panitumumab(L)-(GGGGS)3-SIRPD1-Fc2
DIQMTQSPSSLSASVGDRVTITCQASQDISNYLNWYQQKPGKAPKLLIYDASNLETGVPSRFSGSGSGTDFTFTISSLQPEDIATYFCQHFDHLPLAFGGGTKVEIKRTVAAPSVFIFPPSDEQLKSGTASVVCLLNNFYPREAKVQWKVDNALQSGNSQESVTEQDSKDSTYSLSSTLTLSKADYEKHKVYACEVTHQGLSSPVTKSFNRGECGGGGSGGGGSGGGGSEEELQVIQPDKSVSVAAGESAILHCTVTSLIPVGPIQWFRGAGPARELIYNQKEGHFPRVTTVSESTKRENMDFSISISAITPADAGTYYCVKFRKGSPDTEFKSGAGTELSVRAKPDKTHTCPPCPAPELLGGPSVFLFPPKPKDTLMISRTPEVTCVVVDVSHEDPEVKFNWYVDGVEVHNAKTKPREEQYNSTYRVVSVLTVLHQDWLNGKEYKCKVSNKALPAPIEKTISKAKGQPREPQVYTLPPSRDELTKNQVSLWCLVKGFYPSDIAVEWESNGQPENNYKTTPPVLDSDGSFFLYSKLTVDKSRWQQGNVFSCSVMHEALHNHYTQKSLSLSPGK

SEQ ID NO: 58 - protein, 448 aa, Artificial Sequence
  Tacatuzumab(H)-Fc1
QVQLQQSGAEVKKPGSSVKVSCKASGYAFTSYVIHWVRQAPGQGLYWIGYIHPYNGGTKYNEKFKGKATITADESTNTAYMELSSLRSEDTAFYFCARSGGGDPFAYWGQGSLVTVSSASTKGPSVFPLAPSSKSTSGGTAALGCLVKDYFPEPVTVSWNSGALTSGVHTFPAVLQSSGLYSLSSVVTVPSSSLGTQTYICNVNHKPSNTKVDKRVEPKSCDKTHTCPPCPAPELLGGPSVFLFPPKPKDTLMISRTPEVTCVVVDVSHEDPEVKFNWYVDGVEVHNAKTKPREEQYNSTYRVVSVLTVLHQDWLNGKEYKCKVSNKALPAPIEKTISKAKGQPREPQVYTLPPSRDELTKNQVSLSCAVKGFYPSDIAVEWESNGQPENNYKTTPPVLDSDGSFFLVSKLTVDKSRWQQGNVFSCSVMHEALHNHYTQKSLSLSPGK

SEQ ID NO: 59 - protein, 620 aa, Artificial Sequence
  Tacatuzumab(L)-(GGGGS)3-IFN 2b-Fc2
DIQLTQSPSSLSASVGDRVTITCKASQDINKYIGWYQQKPGKAPKLLMHYTSALLPGIPSRFSGSGSGRDYTFTISSLQPEDIATYYCLQYDDLWTFGGGTKLQIKRTVAAPSVFIFPPSDEQLKSGTASVVCLLNNFYPREAKVQWKVDNALQSGNSQESVTEQDSKDSTYSLSSTLTLSKADYEKHKVYACEVTHQGLSSPVTKSFNRGECGGGGSGGGGSGGGGSCDLPQTHSLGSRRTLMLLAQMRRISLFSCLKDRHDFGFPQEEFGNQFQKAETIPVLHEMIQQIFNLFSTKDSSAAWDETLLDKFYTELYQQLNDLEACVIQGVGVTETPLMKEDSILAVRKYFQRITLYLKEKKYSPCAWEVVRAEIMRSFSLSTNLQESLRSKEDKTHTCPPCPAPELLGGPSVFLFPPKPKDTLMISRTPEVTCVVVDVSHEDPEVKFNWYVDGVEVHNAKTKPREEQYNSTYRVVSVLTVLHQDWLNGKEYKCKVSNKALPAPIEKTISKAKGQPREPQVYTLPPSRDELTKNQVSLWCLVKGFYPSDIAVEWESNGQPENNYKTTPPVLDSDGSFFLYSKLTVDKSRWQQGNVFSCSVMHEALHNHYTQKSLSLSPGK

SEQ ID NO: 60 - protein, 621 aa, Artificial Sequence
  Tacatuzumab(L)-(GGGGS)3-IFN-Fc2
DIQLTQSPSSLSASVGDRVTITCKASQDINKYIGWYQQKPGKAPKLLMHYTSALLPGIPSRFSGSGSGRDYTFTISSLQPEDIATYYCLQYDDLWTFGGGTKLQIKRTVAAPSVFIFPPSDEQLKSGTASVVCLLNNFYPREAKVQWKVDNALQSGNSQESVTEQDSKDSTYSLSSTLTLSKADYEKHKVYACEVTHQGLSSPVTKSFNRGECGGGGSGGGGSGGGGSMSYNLLGFLQRSSNFQCQKLLWQLNGRLEYCLKDRMNFDIPEEIKQLQQFQKEDAALTIYEMLQNIFAIFRQDSSSTGWNETIVENLLANVYHQINHLKTVLEEKLEKEDFTRGKLMSSLHLKRYYGRILHYLKAKEYSHCAWTIVRVEILRNFYFINRLTGYLRNDKTHTCPPCPAPELLGGPSVFLFPPKPKDTLMISRTPEVTCVVVDVSHEDPEVKFNWYVDGVEVHNAKTKPREEQYNSTYRVVSVLTVLHQDWLNGKEYKCKVSNKALPAPIEKTISKAKGQPREPQVYTLPPSRDELTKNQVSLWCLVKGFYPSDIAVEWESNGQPENNYKTTPPVLDSDGSFFLYSKLTVDKSRWQQGNVFSCSVMHEALHNHYTQKSLSLSPGK

SEQ ID NO: 61 - protein, 581 aa, Artificial Sequence
  Ofatumumab(H)-(GGGS)3-SIRPD1-Fc1
EVQLVESGGGLVQPGRSLRLSCAASGFTFNDYAMHWVRQAPGKGLEWVSTISWNSGSIGYADSVKGRFTISRDNAKKSLYLQMNSLRAEDTALYYCAKDIQYGNYYYGMDVWGQGTTVTVSSASTKGPSVFPLAPSSKSTSGGTAALGCLVKDYFPEPVTVSWNSGALTSGVHTFPAVLQSSGLYSLSSVVTVPSSSLGTQTYICNVNHKPSNTKVDKKVEPKSCGGGSGGGSGGGSEEELQVIQPDKSVSVAAGESAILHCTVTSLIPVGPIQWFRGAGPARELIYNQKEGHFPRVTTVSESTKRENMDFSISISAITPADAGTYYCVKFRKGSPDTEFKSGAGTELSVRAKPDKTHTCPPCPAPELLGGPSVFLFPPKPKDTLMISRTPEVTCVVVDVSHEDPEVKFNWYVDGVEVHNAKTKPREEQYNSTYRVVSVLTVLHQDWLNGKEYKCKVSNKALPAPIEKTISKAKGQPREPQVYTLPPSRDELTKNQVSLSCAVKGFYPSDIAVEWESNGQPENNYKTTPPVLDSDGSFFLVSKLTVDKSRWQQGNVFSCSVMHEALHNHYTQKSLSLSPGK

SEQ ID NO: 62 - protein, 441 aa, Artificial Sequence
  Ofatumumab(L)-Fc2
EIVLTQSPATLSLSPGERATLSCRASQSVSSYLAWYQQKPGQAPRLLIYDASNRATGIPARFSGSGSGTDFTLTISSLEPEDFAVYYCQQRSNWPITFGQGTRLEIKRTVAAPSVFIFPPSDEQLKSGTASVVCLLNNFYPREAKVQWKVDNALQSGNSQESVTEQDSKDSTYSLSSTLTLSKADYEKHKVYACEVTHQGLSSPVTKSFNRGECDKTHTCPPCPAPELLGGPSVFLFPPKPKDTLMISRTPEVTCVVVDVSHEDPEVKFNWYVDGVEVHNAKTKPREEQYNSTYRVVSVLTVLHQDWLNGKEYKCKVSNKALPAPIEKTISKAKGQPREPQVYTLPPSRDELTKNQVSLWCLVKGFYPSDIAVEWESNGQPENNYKTTPPVLDSDGSFFLYSKLTVDKSRWQQGNVFSCSVMHEALHNHYTQKSLSLSPGK

SEQ ID NO: 63 - protein, 456 aa, Artificial Sequence
  Tiragolumab(H)-Fc
EVQLQQSGPGLVKPSQTLSLTCAISGDSVSSNSAAWNWIRQSPSRGLEWLGKTYYRFKWYSDYAVSVKGRITINPDTSKNQFSLQLNSVTPEDTAVFYCTRESTTYDLLAGPFDYWGQGTLVTVSSASTKGPSVFPLAPSSKSTSGGTAALGCLVKDYFPEPVTVSWNSGALTSGVHTFPAVLQSSGLYSLSSVVTVPSSSLGTQTYICNVNHKPSNTKVDKKVEPKSCDKTHTCPPCPAPELLGGPSVFLFPPKPKDTLMISRTPEVTCVVVDVSHEDPEVKFNWYVDGVEVHNAKTKPREEQYNSTYRVVSVLTVLHQDWLNGKEYKCKVSNKALPAPIEKTISKAKGQPREPQVYTLPPSREEMTKNQVSLTCLVKGFYPSDIAVEWESNGQPENNYKTTPPVLDSDGSFFLYSKLTVDKSRWQQGNVFSCSVMHEALHNHYTQKSLSLSPGK

SEQ ID NO: 64 - protein, 220 aa, Artificial Sequence
  Tiragolumab (L)
DIVMTQSPDSLAVSLGERATINCKSSQTVLYSSNNKKYLAWYQQKPGQPPNLLIYWASTRESGVPDRFSGSGSGTDFTLTISSLQAEDVAVYYCQQYYSTPFTFGPGTKVEIKRTVAAPSVFIFPPSDEQLKSGTASVVCLLNNFYPREAKVQWKVDNALQSGNSQESVTEQDSKDSTYSLSSTLTLSKADYEKHKVYACEVTHQGLSSPVTKSFNRGEC